European Patent Application EP 4 736 848 A1, published May 6, 2026. Title: 一种含有阳离子脂质的药物组合物及其用途. Applicant: 上海瑞宏迪医药有限公司. The sequence listing filed with the application follows.

SEQUENCE LISTING (26 sequences)

SEQ ID NO: 1 - protein, 623 aa, Homo sapiens
MGTVNKPVVGVLMGFGIITGTLRITNPVRASVLRYDDFHIDEDKLDTNSVYEPYYHSDHAESSWVNRGESSRKAYDHNSPYIWPRNDYDGFLENAHEHHGVYNQGRGIDSGERLMQPTQMSAQEDLGDDTGIHVIPTLNGDDRHKIVNVDQRQYGDVFKGDLNPKPQGQRLIEVSVEENHPFTLRAPIQRIYGVRYTETWSFLPSLTCTGDAAPAIQHICLKHTTCFQDVVVDVDCAENTKEDQLAEISYRFQGKKEADQPWIVVNTSTLFDELELDPPEIEPGVLKVLRTEKQYLGVYIWNMRGSDGTSTYATFLVTWKGDEKTRNPTPAVTPQPRGAEFHMWNYHSHVFSVGDTFSLAMHLQYKIHEAPFDLLLEWLYVPIDPTCQPMRLYSTCLYHPNAPQCLSHMNSGCTFTSPHLAQRVASTVYQNCEHADNYTAYCLGISHMEPSFGLILHDGGTTLKFVDTPESLSGLYVFVVYFNGHVEAVAYTVVSTVDHFVNAIEERGFPPTAGQPPATTKPKEITPVNPGTSPLLRYAAWTGGLAAVVLLCLVIFLICTAKRMRVKAYRVDKSPYNQSMYYAGLPVDDFEDSESTDTEEEFGNAIGGSHGGSSYTVYIDKTR

SEQ ID NO: 2 - DNA, 1872 bp, Homo sapiens
  source 1..1872: mol_type = other DNA
atggggacagttaataaacctgtggtgggggtattgatggggttcggaattatcacgggaacgttgcgtataacgaatccggtcagagcatccgtcttgcgatacgatgattttcacatcgatgaagacaaactggatacaaactccgtatatgagccttactaccattcagatcatgcggagtcttcatgggtaaatcggggagagtcttcgcgaaaagcgtacgatcataactcaccttatatatggccacgtaatgattatgatggatttttagagaacgcacacgaacaccatggggtgtataatcagggccgtggtatcgatagcggggaacggttaatgcaacccacacaaatgtctgcacaggaggatcttggggacgatacgggcatccacgttatccctacgttaaacggcgatgacagacataaaattgtaaatgtggaccaacgtcaatacggtgacgtgtttaaaggagatcttaatccaaaaccccaaggccaaagactcattgaggtgtcagtggaagaaaatcacccgtttactttacgcgcaccgattcagcggatttatggagtccggtacaccgagacttggagctttttgccgtcattaacctgtacgggagacgcagcgcccgccatccagcatatatgtttaaaacatacaacatgctttcaagacgtggtggtggatgtggattgcgcggaaaatactaaagaggatcagttggccgaaatcagttaccgttttcaaggtaagaaggaagcggaccaaccgtggattgttgtaaacacgagcacactgtttgatgaactcgaattagacccccccgagattgaaccgggtgtcttgaaagtacttcggacagaaaaacaatacttgggtgtgtacatttggaacatgcgcggctccgatggtacgtctacctacgccacgtttttggtcacctggaaaggggatgaaaaaacaagaaaccctacgcccgcagtaactcctcaaccaagaggggctgagtttcatatgtggaattaccactcgcatgtattttcagttggtgatacgtttagcttggcaatgcatcttcagtataagatacatgaagcgccatttgatttgctgttagagtggttgtatgtccccatcgatcctacatgtcaaccaatgcggttatattctacgtgtttgtatcatcccaacgcaccccaatgcctctctcatatgaattccggttgtacatttacctcgccacatttagcccagcgtgttgcaagcacagtgtatcaaaattgtgaacatgcagataactacaccgcatattgtctgggaatatctcatatggagcctagctttggtctaatcttacacgacgggggcaccacgttaaagtttgtagatacacccgagagtttgtcgggattatacgtttttgtggtgtattttaacgggcatgttgaagccgtagcatacactgttgtatccacagtagatcattttgtaaacgcaattgaagagcgtggatttccgccaacggccggtcagccaccggcgactactaaacccaaggaaattacccccgtaaaccccggaacgtcaccacttctacgatatgccgcatggaccggagggcttgcagcagtagtacttttatgtctcgtaatatttttaatctgtacggctaaacgaatgagggttaaagcctatagggtagacaagtccccgtataaccaaagcatgtattacgctggccttccagtggacgatttcgaggactcggaatctacggatacggaagaagagtttggtaacgcgattggagggagtcacgggggttcgagttacacggtgtatatagataagacccggtga

SEQ ID NO: 3 - RNA, 1641 nt, synthetic construct
  source 1..1641: mol_type = other RNA; note = gE1
atgggcaccgtgaacaagcccgtggtgggcgtgctgatgggcttcggcatcatcaccggcaccctgcgcatcaccaaccccgtgcgggccagcgtgctgcgctacgacgacttccacatcgacgaggacaagctggacaccaactccgtgtacgagccctactaccacagcgaccacgccgagtccagctgggtgaaccggggcgagtccagccgcaaggcctacgaccacaactccccctacatctggccccggaacgactacgacggcttcctggagaacgcccacgagcaccacggggtgtacaaccagggccgcgggatcgacagcggcgagcggctgatgcagcccacccagatgtccgcccaggaggacctgggggacgacaccggcatccacgtgatccccaccctgaacggggacgaccgccacaagatcgtgaacgtggaccagcggcagtacggcgacgtgttcaagggggacctgaaccccaagccccagggccagcgcctgatcgaggtcagcgtggaggagaaccaccccttcaccctgcgggcccccatccagcgcatctacggggtccggtacaccgagacctggtccttcctgcccagcctgacctgcaccggcgacgccgcccccgccatccagcacatctgcctgaagcacaccacctgcttccaggacgtggtcgtggacgtcgactgcgccgagaacaccaaggaggaccagctcgccgagatctcctaccgcttccaggggaagaaggaggccgaccagccctggatcgtggtcaacaccagcaccctgttcgacgagctggagctggacccgcccgagatcgagcccggcgtgctcaaggtcctgcggaccgagaagcagtacctcggggtgtacatctggaacatgcgcggctccgacgggaccagcacctacgccaccttcctggtcacctggaagggcgacgagaagacccggaaccccacccccgccgtgacgccccagccgcgcggggccgagttccacatgtggaactaccactcccacgtcttcagcgtgggcgacacgttctccctcgccatgcacctgcagtacaagatccacgaggccccgttcgacctcctgctggagtggctgtacgtccccatcgacccgacctgccagcccatgcggctctacagcacgtgcctgtaccaccccaacgccccgcagtgcctctcccacatgaacagcgggtgcaccttcacgtccccgcacctggcgcagcgcgtggccagcaccgtctaccagaactgcgagcacgcggacaactacaccgcctactgcctcggcatctcccacatggagccctcgttcgggctgatcctccacgacggcgggacgaccctgaagttcgtggacacgccggagagcctctccggcctgtacgtcttcgtggtctacttcaacgggcacgtggaggcggtcgcctacacggtggtctcgaccgtggaccacttcgtcaacgcgatcgaggagcggggctttcccccgaccgccgggcagccgcccgcgacgacgaagccgaaggagatcaccccggtgaaccccggcacgagcccgctcctgcgctacgccgcgtggaccgggggcctcgcctga

SEQ ID NO: 4 - RNA, 1725 nt, synthetic construct
  source 1..1725: mol_type = other RNA; note = gE2
atgggcaccgtgaacaagcccgtggtgggcgtgctgatgggcttcggcatcatcaccggcaccctgcgcatcaccaaccccgtgcgggccagcgtgctgcgctacgacgacttccacatcgacgaggacaagctggacaccaactccgtgtacgagccctactaccacagcgaccacgccgagtccagctgggtgaaccggggcgagtccagccgcaaggcctacgaccacaactccccctacatctggccccggaacgactacgacggcttcctggagaacgcccacgagcaccacggggtgtacaaccagggccgcgggatcgacagcggcgagcggctgatgcagcccacccagatgtccgcccaggaggacctgggggacgacaccggcatccacgtgatccccaccctgaacggggacgaccgccacaagatcgtgaacgtggaccagcggcagtacggcgacgtgttcaagggggacctgaaccccaagccccagggccagcgcctgatcgaggtcagcgtggaggagaaccaccccttcaccctgcgggcccccatccagcgcatctacggggtccggtacaccgagacctggtccttcctgcccagcctgacctgcaccggcgacgccgcccccgccatccagcacatctgcctgaagcacaccacctgcttccaggacgtggtcgtggacgtcgactgcgccgagaacaccaaggaggaccagctcgccgagatctcctaccgcttccaggggaagaaggaggccgaccagccctggatcgtggtcaacaccagcaccctgttcgacgagctggagctggacccgcccgagatcgagcccggcgtgctcaaggtcctgcggaccgagaagcagtacctcggggtgtacatctggaacatgcgcggctccgacgggaccagcacctacgccaccttcctggtcacctggaagggcgacgagaagacccggaaccccacccccgccgtgacgccccagccgcgcggggccgagttccacatgtggaactaccactcccacgtcttcagcgtgggcgacacgttctccctcgccatgcacctgcagtacaagatccacgaggccccgttcgacctcctgctggagtggctgtacgtccccatcgacccgacctgccagcccatgcggctctacagcacgtgcctgtaccaccccaacgccccgcagtgcctctcccacatgaacagcgggtgcaccttcacgtccccgcacctggcgcagcgcgtggccagcaccgtctaccagaactgcgagcacgcggacaactacaccgcctactgcctcggcatctcccacatggagccctcgttcgggctgatcctccacgacggcgggacgaccctgaagttcgtggacacgccggagagcctctccggcctgtacgtcttcgtggtctacttcaacgggcacgtggaggcggtcgcctacacggtggtctcgaccgtggaccacttcgtcaacgcgatcgaggagcggggctttcccccgaccgccgggcagccgcccgcgacgacgaagccgaaggagatcaccccggtgaaccccggcacgagcccgctcctgcgctacgccgcgtggaccgggggcctcgccgcggtcgtgctgctctgcctggtcatcttcctcatctgcaccgccaagcggatgcgcgtgaaggcggcccgggtcgacaagtcctga

SEQ ID NO: 5 - RNA, 1635 nt, synthetic construct
  source 1..1635: mol_type = other RNA; note = gE3
atgggcaccgtgaacaagcccgtggtgggcgtgctgatgggcttcggcatcatcaccggcaccctgcgcatcaccaaccccgtgcgggccagcgtgctgcgctacgacgacttccacatcgacgaggacaagctggacaccaactccgtgtacgagccctactaccacagcgaccacgccgagtccagctgggtgaaccggggcgagtccagccgcaaggcctacgaccacaactccccctacatctggccccggaacgactacgacggcttcctggagaacgcccacgagcaccacggggtgtacaaccagggccgcgggatcgacagcggcgagcggctgatgcagcccacccagatgtccgcccaggaggacctgggggacgacaccggcatccacgtgatccccaccctgaacggggacgaccgccacaagatcgtgaacgtggaccagcggcagtacggcgacgtgttcaagggggacctgaaccccaagccccagggccagcgcctgatcgaggtcagcgtggaggagaaccaccccttcaccctgcgggcccccatccagcgcatctacggggtccggtacaccgagacctggtccttcctgcccagcctgacctgcaccggcgacgccgcccccgccatccagcacatctgcctgaagcacaccacctgcttccaggacgtggtcgtggacgtcgactgcgccgagaacaccaaggaggaccagctcgccgagatctcctaccgcttccaggggaagaaggaggccgaccagccctggatcgtggtcaacaccagcaccctgttcgacgagctggagctggacccgcccgagatcgagcccggcgtgctcaaggtcctgcggaccgagaagcagtacctcggggtgtacatctggaacatgcgcggctccgacgggaccagcacctacgccaccttcctggtcacctggaagggcgacgagaagacccggaaccccacccccgccgtgacgccccagccgcgcggggccgagttccacatgtggaactaccactcccacgtcttcagcgtgggcgacacgttctccctcgccatgcacctgcagtacaagatccacgaggccccgttcgacctcctgctggagtggctgtacgtccccatcgacccgacctgccagcccatgcggctctacagcacgtgcctgtaccaccccaacgccccgcagtgcctctcccacatgaacagcgggtgcaccttcacgtccccgcacctggcgcagcgcgtggccagcaccgtctaccagaactgcgagcacgcggacaactacaccgcctactgcctcggcatctcccacatggagccctcgttcgggctgatcctccacgacggcgggacgaccctgaagttcgtggacacgccggagagcctctccggcctgtacgtcttcgtggtctacttcaacgggcacgtggaggcggtcgcctacacggtggtctcgaccgtggaccacttcgtcaacgcgatcgaggagcggggctttcccccgaccgccgggcagccgcccgcgacgacgaagccgaaggagatcaccccggtgaaccccggcacgagcccgctcctgcgctacgccgcgtggaccgggggctga

SEQ ID NO: 6 - RNA, 1725 nt, synthetic construct
  source 1..1725: mol_type = other RNA; note = gE4
atgggcaccgtgaacaagcccgtggtgggcgtgctgatgggcttcggcatcatcaccggcaccctgcgcatcaccaaccccgtgcgggccagcgtgctgcgctacgacgacttccacatcgacgaggacaagctggacaccaactccgtgtacgagccctactaccacagcgaccacgccgagtccagctgggtgaaccggggcgagtccagccgcaaggcctacgaccacaactccccctacatctggccccggaacgactacgacggcttcctggagaacgcccacgagcaccacggggtgtacaaccagggccgcgggatcgacagcggcgagcggctgatgcagcccacccagatgtccgcccaggaggacctgggggacgacaccggcatccacgtgatccccaccctgaacggggacgaccgccacaagatcgtgaacgtggaccagcggcagtacggcgacgtgttcaagggggacctgaaccccaagccccagggccagcgcctgatcgaggtcagcgtggaggagaaccaccccttcaccctgcgggcccccatccagcgcatctacggggtccggtacaccgagacctggtccttcctgcccagcctgacctgcaccggcgacgccgcccccgccatccagcacatctgcctgaagcacaccacctgcttccaggacgtggtcgtggacgtcgactgcgccgagaacaccaaggaggaccagctcgccgagatctcctaccgcttccaggggaagaaggaggccgaccagccctggatcgtggtcaacaccagcaccctgttcgacgagctggagctggacccgcccgagatcgagcccggcgtgctcaaggtcctgcggaccgagaagcagtacctcggggtgtacatctggaacatgcgcggctccgacgggaccagcacctacgccaccttcctggtcacctggaagggcgacgagaagacccggaaccccacccccgccgtgacgccccagccgcgcggggccgagttccacatgtggaactaccactcccacgtcttcagcgtgggcgacacgttctccctcgccatgcacctgcagtacaagatccacgaggccccgttcgacctcctgctggagtggctgtacgtccccatcgacccgacctgccagcccatgcggctctacagcacgtgcctgtaccaccccaacgccccgcagtgcctctcccacatgaacagcgggtgcaccttcacgtccccgcacctggcgcagcgcgtggccagcaccgtctaccagaactgcgagcacgcggacaactacaccgcctactgcctcggcatctcccacatggagccctcgttcgggctgatcctccacgacggcgggacgaccctgaagttcgtggacacgccggagagcctctccggcctgtacgtcttcgtggtctacttcaacgggcacgtggaggcggtcgcctacacggtggtctcgaccgtggaccacttcgtcaacgcgatcgaggagcggggctttcccccgaccgccgggcagccgcccgcgacgacgaagccgaaggagatcaccccggtgaaccccggcacgagcccgctcctgcgctacgccgcgtggaccgggggcctcgccgcggtcgtgctgctctgcctggtcatcttcctcatctgcaccgccaagcggatgcgcgtgaaggcgtaccgggtcgacaagtcctga

SEQ ID NO: 7 - RNA, 1686 nt, synthetic construct
  source 1..1686: mol_type = other RNA; note = gE5
atgggcaccgtgaacaagcccgtggtgggcgtgctgatgggcttcggcatcatcaccggcaccctgcgcatcaccaaccccgtgcgggccagcgtgctgcgctacgacgacttccacatcgacgaggacaagctggacaccaactccgtgtacgagccctactaccacagcgaccacgccgagtccagctgggtgaaccggggcgagtccagccgcaaggcctacgaccacaactccccctacatctggccccggaacgactacgacggcttcctggagaacgcccacgagcaccacggggtgtacaaccagggccgcgggatcgacagcggcgagcggctgatgcagcccacccagatgtccgcccaggaggacctgggggacgacaccggcatccacgtgatccccaccctgaacggggacgaccgccacaagatcgtgaacgtggaccagcggcagtacggcgacgtgttcaagggggacctgaaccccaagccccagggccagcgcctgatcgaggtcagcgtggaggagaaccaccccttcaccctgcgggcccccatccagcgcatctacggggtccggtacaccgagacctggtccttcctgcccagcctgacctgcaccggcgacgccgcccccgccatccagcacatctgcctgaagcacaccacctgcttccaggacgtggtcgtggacgtcgactgcgccgagaacaccaaggaggaccagctcgccgagatctcctaccgcttccaggggaagaaggaggccgaccagccctggatcgtggtcaacaccagcaccctgttcgacgagctggagctggacccgcccgagatcgagcccggcgtgctcaaggtcctgcggaccgagaagcagtacctcggggtgtacatctggaacatgcgcggctccgacgggaccagcacctacgccaccttcctggtcacctggaagggcgacgagaagacccggaaccccacccccgccgtgacgccccagccgcgcggggccgagttccacatgtggaactaccactcccacgtcttcagcgtgggcgacacgttctccctcgccatgcacctgcagtacaagatccacgaggccccgttcgacctcctgctggagtggctgtacgtccccatcgacccgacctgccagcccatgcggctctacagcacgtgcctgtaccaccccaacgccccgcagtgcctctcccacatgaacagcgggtgcaccttcacgtccccgcacctggcgcagcgcgtggccagcaccgtctaccagaactgcgagcacgcggacaactacaccgcctactgcctcggcatctcccacatggagccctcgttcgggctgatcctccacgacggcgggacgaccctgaagttcgtggacacgccggagagcctctccggcctgtacgtcttcgtggtctacttcaacgggcacgtggaggcggtcgcctacacggtggtctcgaccgtggaccacttcgtcaacgcgatcgaggagcggggctttcccccgaccgccgggcagccgcccgcgacgacgaagccgaaggagatcaccccggtgaaccccggcacgagcccgctcctgcgctacgccgcgtggaccgggggcctcgccgcggtcgtgctgctctgcctggtcatcttcctcatctgcaccgcctga

SEQ ID NO: 8 - RNA, 1872 nt, synthetic construct
  source 1..1872: mol_type = other RNA; note = gE6
atgggcaccgtgaacaagcccgtggtgggcgtgctgatgggcttcggcatcatcaccggcaccctgcgcatcaccaaccccgtgcgggccagcgtgctgcgctacgacgacttccacatcgacgaggacaagctggacaccaactccgtgtacgagccctactaccacagcgaccacgccgagtccagctgggtgaaccggggcgagtccagccgcaaggcctacgaccacaactccccctacatctggccccggaacgactacgacggcttcctggagaacgcccacgagcaccacggggtgtacaaccagggccgcgggatcgacagcggcgagcggctgatgcagcccacccagatgtccgcccaggaggacctgggggacgacaccggcatccacgtgatccccaccctgaacggggacgaccgccacaagatcgtgaacgtggaccagcggcagtacggcgacgtgttcaagggggacctgaaccccaagccccagggccagcgcctgatcgaggtcagcgtggaggagaaccaccccttcaccctgcgggcccccatccagcgcatctacggggtccggtacaccgagacctggtccttcctgcccagcctgacctgcaccggcgacgccgcccccgccatccagcacatctgcctgaagcacaccacctgcttccaggacgtggtcgtggacgtcgactgcgccgagaacaccaaggaggaccagctcgccgagatctcctaccgcttccaggggaagaaggaggccgaccagccctggatcgtggtcaacaccagcaccctgttcgacgagctggagctggacccgcccgagatcgagcccggcgtgctcaaggtcctgcggaccgagaagcagtacctcggggtgtacatctggaacatgcgcggctccgacgggaccagcacctacgccaccttcctggtcacctggaagggcgacgagaagacccggaaccccacccccgccgtgacgccccagccgcgcggggccgagttccacatgtggaactaccactcccacgtcttcagcgtgggcgacacgttctccctcgccatgcacctgcagtacaagatccacgaggccccgttcgacctcctgctggagtggctgtacgtccccatcgacccgacctgccagcccatgcggctctacagcacgtgcctgtaccaccccaacgccccgcagtgcctctcccacatgaacagcgggtgcaccttcacgtccccgcacctggcgcagcgcgtggccagcaccgtctaccagaactgcgagcacgcggacaactacaccgcctactgcctcggcatctcccacatggagccctcgttcgggctgatcctccacgacggcgggacgaccctgaagttcgtggacacgccggagagcctctccggcctgtacgtcttcgtggtctacttcaacgggcacgtggaggcggtcgcctacacggtggtctcgaccgtggaccacttcgtcaacgcgatcgaggagcggggctttcccccgaccgccgggcagccgcccgcgacgacgaagccgaaggagatcaccccggtgaaccccggcacgagcccgctcctgcgctacgccgcgtggaccgggggcctcgccgcggtcgtgctgctctgcctggtcatcttcctcatctgcaccgccaagcggatgcgcgtgaaggcgtaccgggtcgacaagtccccctacaaccagtcgatgtactacgccgggctgcccgtggacgacttcgaggacagcgagtccacggacaccgaggaggagttcggcaacgcgatcgggggctcgcacgggggctcctcgtacacggtctacatcgacaagacccgctga

SEQ ID NO: 9 - RNA, 63 nt, synthetic construct
  source 1..63: mol_type = other RNA; note = 5'UTR
gagttaggagttggtggcagtttcaataacaggtcattgccgagaaaaggatagcactataat

SEQ ID NO: 10 - RNA, 134 nt, synthetic construct
  source 1..134: mol_type = other RNA; note = 3'UTR
gctcgctttcttgctgtccaatttctattaaaggttcctttgttccctaagtccaactactaaactgggggatattatgaagggccttgagcatctggattctgcctaataaaaaacatttattttcattgcaa

SEQ ID NO: 11 - RNA, 110 nt, synthetic construct
  source 1..110: mol_type = other RNA; note = 30L70A polyA
aaaaaaaaaaaaaaaaaaaaaaaaaaaaaagcatatgactaaaaaaaaaaaaaaaaaaaaaaaaaaaaaaaaaaaaaaaaaaaaaaaaaaaaaaaaaaaaaaaaaaaaaa

SEQ ID NO: 12 - RNA, 120 nt, synthetic construct
  source 1..120: mol_type = other RNA; note = 120A polyA
aaaaaaaaaaaaaaaaaaaaaaaaaaaaaaaaaaaaaaaaaaaaaaaaaaaaaaaaaaaaaaaaaaaaaaaaaaaaaaaaaaaaaaaaaaaaaaaaaaaaaaaaaaaaaaaaaaaaaaaa

SEQ ID NO: 13 - RNA, 1957 nt, synthetic construct
  source 1..1957: mol_type = other RNA; note = gE1 (30L70A) mRNA
gagttaggagttggtggcagtttcaataacaggtcattgccgagaaaaggatagcactataatatgggcaccgtgaacaagcccgtggtgggcgtgctgatgggcttcggcatcatcaccggcaccctgcgcatcaccaaccccgtgcgggccagcgtgctgcgctacgacgacttccacatcgacgaggacaagctggacaccaactccgtgtacgagccctactaccacagcgaccacgccgagtccagctgggtgaaccggggcgagtccagccgcaaggcctacgaccacaactccccctacatctggccccggaacgactacgacggcttcctggagaacgcccacgagcaccacggggtgtacaaccagggccgcgggatcgacagcggcgagcggctgatgcagcccacccagatgtccgcccaggaggacctgggggacgacaccggcatccacgtgatccccaccctgaacggggacgaccgccacaagatcgtgaacgtggaccagcggcagtacggcgacgtgttcaagggggacctgaaccccaagccccagggccagcgcctgatcgaggtcagcgtggaggagaaccaccccttcaccctgcgggcccccatccagcgcatctacggggtccggtacaccgagacctggtccttcctgcccagcctgacctgcaccggcgacgccgcccccgccatccagcacatctgcctgaagcacaccacctgcttccaggacgtggtcgtggacgtcgactgcgccgagaacaccaaggaggaccagctcgccgagatctcctaccgcttccaggggaagaaggaggccgaccagccctggatcgtggtcaacaccagcaccctgttcgacgagctggagctggacccgcccgagatcgagcccggcgtgctcaaggtcctgcggaccgagaagcagtacctcggggtgtacatctggaacatgcgcggctccgacgggaccagcacctacgccaccttcctggtcacctggaagggcgacgagaagacccggaaccccacccccgccgtgacgccccagccgcgcggggccgagttccacatgtggaactaccactcccacgtcttcagcgtgggcgacacgttctccctcgccatgcacctgcagtacaagatccacgaggccccgttcgacctcctgctggagtggctgtacgtccccatcgacccgacctgccagcccatgcggctctacagcacgtgcctgtaccaccccaacgccccgcagtgcctctcccacatgaacagcgggtgcaccttcacgtccccgcacctggcgcagcgcgtggccagcaccgtctaccagaactgcgagcacgcggacaactacaccgcctactgcctcggcatctcccacatggagccctcgttcgggctgatcctccacgacggcgggacgaccctgaagttcgtggacacgccggagagcctctccggcctgtacgtcttcgtggtctacttcaacgggcacgtggaggcggtcgcctacacggtggtctcgaccgtggaccacttcgtcaacgcgatcgaggagcggggctttcccccgaccgccgggcagccgcccgcgacgacgaagccgaaggagatcaccccggtgaaccccggcacgagcccgctcctgcgctacgccgcgtggaccgggggcctcgcctgatgaaccggtgctcgctttcttgctgtccaatttctattaaaggttcctttgttccctaagtccaactactaaactgggggatattatgaagggccttgagcatctggattctgcctaataaaaaacatttattttcattgcaaaaaaaaaaaaaaaaaaaaaaaaaaaaaaaagcatatgactaaaaaaaaaaaaaaaaaaaaaaaaaaaaaaaaaaaaaaaaaaaaaaaaaaaaaaaaaaaaaaaaaaaaaa

SEQ ID NO: 14 - RNA, 2041 nt, synthetic construct
  source 1..2041: mol_type = other RNA; note = gE2 (30L70A) mRNA
gagttaggagttggtggcagtttcaataacaggtcattgccgagaaaaggatagcactataatatgggcaccgtgaacaagcccgtggtgggcgtgctgatgggcttcggcatcatcaccggcaccctgcgcatcaccaaccccgtgcgggccagcgtgctgcgctacgacgacttccacatcgacgaggacaagctggacaccaactccgtgtacgagccctactaccacagcgaccacgccgagtccagctgggtgaaccggggcgagtccagccgcaaggcctacgaccacaactccccctacatctggccccggaacgactacgacggcttcctggagaacgcccacgagcaccacggggtgtacaaccagggccgcgggatcgacagcggcgagcggctgatgcagcccacccagatgtccgcccaggaggacctgggggacgacaccggcatccacgtgatccccaccctgaacggggacgaccgccacaagatcgtgaacgtggaccagcggcagtacggcgacgtgttcaagggggacctgaaccccaagccccagggccagcgcctgatcgaggtcagcgtggaggagaaccaccccttcaccctgcgggcccccatccagcgcatctacggggtccggtacaccgagacctggtccttcctgcccagcctgacctgcaccggcgacgccgcccccgccatccagcacatctgcctgaagcacaccacctgcttccaggacgtggtcgtggacgtcgactgcgccgagaacaccaaggaggaccagctcgccgagatctcctaccgcttccaggggaagaaggaggccgaccagccctggatcgtggtcaacaccagcaccctgttcgacgagctggagctggacccgcccgagatcgagcccggcgtgctcaaggtcctgcggaccgagaagcagtacctcggggtgtacatctggaacatgcgcggctccgacgggaccagcacctacgccaccttcctggtcacctggaagggcgacgagaagacccggaaccccacccccgccgtgacgccccagccgcgcggggccgagttccacatgtggaactaccactcccacgtcttcagcgtgggcgacacgttctccctcgccatgcacctgcagtacaagatccacgaggccccgttcgacctcctgctggagtggctgtacgtccccatcgacccgacctgccagcccatgcggctctacagcacgtgcctgtaccaccccaacgccccgcagtgcctctcccacatgaacagcgggtgcaccttcacgtccccgcacctggcgcagcgcgtggccagcaccgtctaccagaactgcgagcacgcggacaactacaccgcctactgcctcggcatctcccacatggagccctcgttcgggctgatcctccacgacggcgggacgaccctgaagttcgtggacacgccggagagcctctccggcctgtacgtcttcgtggtctacttcaacgggcacgtggaggcggtcgcctacacggtggtctcgaccgtggaccacttcgtcaacgcgatcgaggagcggggctttcccccgaccgccgggcagccgcccgcgacgacgaagccgaaggagatcaccccggtgaaccccggcacgagcccgctcctgcgctacgccgcgtggaccgggggcctcgccgcggtcgtgctgctctgcctggtcatcttcctcatctgcaccgccaagcggatgcgcgtgaaggcggcccgggtcgacaagtcctgatgaaccggtgctcgctttcttgctgtccaatttctattaaaggttcctttgttccctaagtccaactactaaactgggggatattatgaagggccttgagcatctggattctgcctaataaaaaacatttattttcattgcaaaaaaaaaaaaaaaaaaaaaaaaaaaaaaaagcatatgactaaaaaaaaaaaaaaaaaaaaaaaaaaaaaaaaaaaaaaaaaaaaaaaaaaaaaaaaaaaaaaaaaaaaaa

SEQ ID NO: 15 - RNA, 1951 nt, synthetic construct
  source 1..1951: mol_type = other RNA; note = gE3 (30L70A) mRNA
gagttaggagttggtggcagtttcaataacaggtcattgccgagaaaaggatagcactataatatgggcaccgtgaacaagcccgtggtgggcgtgctgatgggcttcggcatcatcaccggcaccctgcgcatcaccaaccccgtgcgggccagcgtgctgcgctacgacgacttccacatcgacgaggacaagctggacaccaactccgtgtacgagccctactaccacagcgaccacgccgagtccagctgggtgaaccggggcgagtccagccgcaaggcctacgaccacaactccccctacatctggccccggaacgactacgacggcttcctggagaacgcccacgagcaccacggggtgtacaaccagggccgcgggatcgacagcggcgagcggctgatgcagcccacccagatgtccgcccaggaggacctgggggacgacaccggcatccacgtgatccccaccctgaacggggacgaccgccacaagatcgtgaacgtggaccagcggcagtacggcgacgtgttcaagggggacctgaaccccaagccccagggccagcgcctgatcgaggtcagcgtggaggagaaccaccccttcaccctgcgggcccccatccagcgcatctacggggtccggtacaccgagacctggtccttcctgcccagcctgacctgcaccggcgacgccgcccccgccatccagcacatctgcctgaagcacaccacctgcttccaggacgtggtcgtggacgtcgactgcgccgagaacaccaaggaggaccagctcgccgagatctcctaccgcttccaggggaagaaggaggccgaccagccctggatcgtggtcaacaccagcaccctgttcgacgagctggagctggacccgcccgagatcgagcccggcgtgctcaaggtcctgcggaccgagaagcagtacctcggggtgtacatctggaacatgcgcggctccgacgggaccagcacctacgccaccttcctggtcacctggaagggcgacgagaagacccggaaccccacccccgccgtgacgccccagccgcgcggggccgagttccacatgtggaactaccactcccacgtcttcagcgtgggcgacacgttctccctcgccatgcacctgcagtacaagatccacgaggccccgttcgacctcctgctggagtggctgtacgtccccatcgacccgacctgccagcccatgcggctctacagcacgtgcctgtaccaccccaacgccccgcagtgcctctcccacatgaacagcgggtgcaccttcacgtccccgcacctggcgcagcgcgtggccagcaccgtctaccagaactgcgagcacgcggacaactacaccgcctactgcctcggcatctcccacatggagccctcgttcgggctgatcctccacgacggcgggacgaccctgaagttcgtggacacgccggagagcctctccggcctgtacgtcttcgtggtctacttcaacgggcacgtggaggcggtcgcctacacggtggtctcgaccgtggaccacttcgtcaacgcgatcgaggagcggggctttcccccgaccgccgggcagccgcccgcgacgacgaagccgaaggagatcaccccggtgaaccccggcacgagcccgctcctgcgctacgccgcgtggaccgggggctgatgaaccggtgctcgctttcttgctgtccaatttctattaaaggttcctttgttccctaagtccaactactaaactgggggatattatgaagggccttgagcatctggattctgcctaataaaaaacatttattttcattgcaaaaaaaaaaaaaaaaaaaaaaaaaaaaaaaagcatatgactaaaaaaaaaaaaaaaaaaaaaaaaaaaaaaaaaaaaaaaaaaaaaaaaaaaaaaaaaaaaaaaaaaaaaa

SEQ ID NO: 16 - RNA, 2041 nt, synthetic construct
  source 1..2041: mol_type = other RNA; note = gE4 (30L70A) mRNA
gagttaggagttggtggcagtttcaataacaggtcattgccgagaaaaggatagcactataatatgggcaccgtgaacaagcccgtggtgggcgtgctgatgggcttcggcatcatcaccggcaccctgcgcatcaccaaccccgtgcgggccagcgtgctgcgctacgacgacttccacatcgacgaggacaagctggacaccaactccgtgtacgagccctactaccacagcgaccacgccgagtccagctgggtgaaccggggcgagtccagccgcaaggcctacgaccacaactccccctacatctggccccggaacgactacgacggcttcctggagaacgcccacgagcaccacggggtgtacaaccagggccgcgggatcgacagcggcgagcggctgatgcagcccacccagatgtccgcccaggaggacctgggggacgacaccggcatccacgtgatccccaccctgaacggggacgaccgccacaagatcgtgaacgtggaccagcggcagtacggcgacgtgttcaagggggacctgaaccccaagccccagggccagcgcctgatcgaggtcagcgtggaggagaaccaccccttcaccctgcgggcccccatccagcgcatctacggggtccggtacaccgagacctggtccttcctgcccagcctgacctgcaccggcgacgccgcccccgccatccagcacatctgcctgaagcacaccacctgcttccaggacgtggtcgtggacgtcgactgcgccgagaacaccaaggaggaccagctcgccgagatctcctaccgcttccaggggaagaaggaggccgaccagccctggatcgtggtcaacaccagcaccctgttcgacgagctggagctggacccgcccgagatcgagcccggcgtgctcaaggtcctgcggaccgagaagcagtacctcggggtgtacatctggaacatgcgcggctccgacgggaccagcacctacgccaccttcctggtcacctggaagggcgacgagaagacccggaaccccacccccgccgtgacgccccagccgcgcggggccgagttccacatgtggaactaccactcccacgtcttcagcgtgggcgacacgttctccctcgccatgcacctgcagtacaagatccacgaggccccgttcgacctcctgctggagtggctgtacgtccccatcgacccgacctgccagcccatgcggctctacagcacgtgcctgtaccaccccaacgccccgcagtgcctctcccacatgaacagcgggtgcaccttcacgtccccgcacctggcgcagcgcgtggccagcaccgtctaccagaactgcgagcacgcggacaactacaccgcctactgcctcggcatctcccacatggagccctcgttcgggctgatcctccacgacggcgggacgaccctgaagttcgtggacacgccggagagcctctccggcctgtacgtcttcgtggtctacttcaacgggcacgtggaggcggtcgcctacacggtggtctcgaccgtggaccacttcgtcaacgcgatcgaggagcggggctttcccccgaccgccgggcagccgcccgcgacgacgaagccgaaggagatcaccccggtgaaccccggcacgagcccgctcctgcgctacgccgcgtggaccgggggcctcgccgcggtcgtgctgctctgcctggtcatcttcctcatctgcaccgccaagcggatgcgcgtgaaggcgtaccgggtcgacaagtcctgatgaaccggtgctcgctttcttgctgtccaatttctattaaaggttcctttgttccctaagtccaactactaaactgggggatattatgaagggccttgagcatctggattctgcctaataaaaaacatttattttcattgcaaaaaaaaaaaaaaaaaaaaaaaaaaaaaaaagcatatgactaaaaaaaaaaaaaaaaaaaaaaaaaaaaaaaaaaaaaaaaaaaaaaaaaaaaaaaaaaaaaaaaaaaaaa

SEQ ID NO: 17 - RNA, 2002 nt, synthetic construct
  source 1..2002: mol_type = other RNA; note = gE5 (30L70A) mRNA
gagttaggagttggtggcagtttcaataacaggtcattgccgagaaaaggatagcactataatatgggcaccgtgaacaagcccgtggtgggcgtgctgatgggcttcggcatcatcaccggcaccctgcgcatcaccaaccccgtgcgggccagcgtgctgcgctacgacgacttccacatcgacgaggacaagctggacaccaactccgtgtacgagccctactaccacagcgaccacgccgagtccagctgggtgaaccggggcgagtccagccgcaaggcctacgaccacaactccccctacatctggccccggaacgactacgacggcttcctggagaacgcccacgagcaccacggggtgtacaaccagggccgcgggatcgacagcggcgagcggctgatgcagcccacccagatgtccgcccaggaggacctgggggacgacaccggcatccacgtgatccccaccctgaacggggacgaccgccacaagatcgtgaacgtggaccagcggcagtacggcgacgtgttcaagggggacctgaaccccaagccccagggccagcgcctgatcgaggtcagcgtggaggagaaccaccccttcaccctgcgggcccccatccagcgcatctacggggtccggtacaccgagacctggtccttcctgcccagcctgacctgcaccggcgacgccgcccccgccatccagcacatctgcctgaagcacaccacctgcttccaggacgtggtcgtggacgtcgactgcgccgagaacaccaaggaggaccagctcgccgagatctcctaccgcttccaggggaagaaggaggccgaccagccctggatcgtggtcaacaccagcaccctgttcgacgagctggagctggacccgcccgagatcgagcccggcgtgctcaaggtcctgcggaccgagaagcagtacctcggggtgtacatctggaacatgcgcggctccgacgggaccagcacctacgccaccttcctggtcacctggaagggcgacgagaagacccggaaccccacccccgccgtgacgccccagccgcgcggggccgagttccacatgtggaactaccactcccacgtcttcagcgtgggcgacacgttctccctcgccatgcacctgcagtacaagatccacgaggccccgttcgacctcctgctggagtggctgtacgtccccatcgacccgacctgccagcccatgcggctctacagcacgtgcctgtaccaccccaacgccccgcagtgcctctcccacatgaacagcgggtgcaccttcacgtccccgcacctggcgcagcgcgtggccagcaccgtctaccagaactgcgagcacgcggacaactacaccgcctactgcctcggcatctcccacatggagccctcgttcgggctgatcctccacgacggcgggacgaccctgaagttcgtggacacgccggagagcctctccggcctgtacgtcttcgtggtctacttcaacgggcacgtggaggcggtcgcctacacggtggtctcgaccgtggaccacttcgtcaacgcgatcgaggagcggggctttcccccgaccgccgggcagccgcccgcgacgacgaagccgaaggagatcaccccggtgaaccccggcacgagcccgctcctgcgctacgccgcgtggaccgggggcctcgccgcggtcgtgctgctctgcctggtcatcttcctcatctgcaccgcctgatgaaccggtgctcgctttcttgctgtccaatttctattaaaggttcctttgttccctaagtccaactactaaactgggggatattatgaagggccttgagcatctggattctgcctaataaaaaacatttattttcattgcaaaaaaaaaaaaaaaaaaaaaaaaaaaaaaaagcatatgactaaaaaaaaaaaaaaaaaaaaaaaaaaaaaaaaaaaaaaaaaaaaaaaaaaaaaaaaaaaaaaaaaaaaaa

SEQ ID NO: 18 - RNA, 2188 nt, synthetic construct
  source 1..2188: mol_type = other RNA; note = gE6 (30L70A) mRNA
gagttaggagttggtggcagtttcaataacaggtcattgccgagaaaaggatagcactataatatgggcaccgtgaacaagcccgtggtgggcgtgctgatgggcttcggcatcatcaccggcaccctgcgcatcaccaaccccgtgcgggccagcgtgctgcgctacgacgacttccacatcgacgaggacaagctggacaccaactccgtgtacgagccctactaccacagcgaccacgccgagtccagctgggtgaaccggggcgagtccagccgcaaggcctacgaccacaactccccctacatctggccccggaacgactacgacggcttcctggagaacgcccacgagcaccacggggtgtacaaccagggccgcgggatcgacagcggcgagcggctgatgcagcccacccagatgtccgcccaggaggacctgggggacgacaccggcatccacgtgatccccaccctgaacggggacgaccgccacaagatcgtgaacgtggaccagcggcagtacggcgacgtgttcaagggggacctgaaccccaagccccagggccagcgcctgatcgaggtcagcgtggaggagaaccaccccttcaccctgcgggcccccatccagcgcatctacggggtccggtacaccgagacctggtccttcctgcccagcctgacctgcaccggcgacgccgcccccgccatccagcacatctgcctgaagcacaccacctgcttccaggacgtggtcgtggacgtcgactgcgccgagaacaccaaggaggaccagctcgccgagatctcctaccgcttccaggggaagaaggaggccgaccagccctggatcgtggtcaacaccagcaccctgttcgacgagctggagctggacccgcccgagatcgagcccggcgtgctcaaggtcctgcggaccgagaagcagtacctcggggtgtacatctggaacatgcgcggctccgacgggaccagcacctacgccaccttcctggtcacctggaagggcgacgagaagacccggaaccccacccccgccgtgacgccccagccgcgcggggccgagttccacatgtggaactaccactcccacgtcttcagcgtgggcgacacgttctccctcgccatgcacctgcagtacaagatccacgaggccccgttcgacctcctgctggagtggctgtacgtccccatcgacccgacctgccagcccatgcggctctacagcacgtgcctgtaccaccccaacgccccgcagtgcctctcccacatgaacagcgggtgcaccttcacgtccccgcacctggcgcagcgcgtggccagcaccgtctaccagaactgcgagcacgcggacaactacaccgcctactgcctcggcatctcccacatggagccctcgttcgggctgatcctccacgacggcgggacgaccctgaagttcgtggacacgccggagagcctctccggcctgtacgtcttcgtggtctacttcaacgggcacgtggaggcggtcgcctacacggtggtctcgaccgtggaccacttcgtcaacgcgatcgaggagcggggctttcccccgaccgccgggcagccgcccgcgacgacgaagccgaaggagatcaccccggtgaaccccggcacgagcccgctcctgcgctacgccgcgtggaccgggggcctcgccgcggtcgtgctgctctgcctggtcatcttcctcatctgcaccgccaagcggatgcgcgtgaaggcgtaccgggtcgacaagtccccctacaaccagtcgatgtactacgccgggctgcccgtggacgacttcgaggacagcgagtccacggacaccgaggaggagttcggcaacgcgatcgggggctcgcacgggggctcctcgtacacggtctacatcgacaagacccgctgatgaaccggtgctcgctttcttgctgtccaatttctattaaaggttcctttgttccctaagtccaactactaaactgggggatattatgaagggccttgagcatctggattctgcctaataaaaaacatttattttcattgcaaaaaaaaaaaaaaaaaaaaaaaaaaaaaaaagcatatgactaaaaaaaaaaaaaaaaaaaaaaaaaaaaaaaaaaaaaaaaaaaaaaaaaaaaaaaaaaaaaaaaaaaaaa

SEQ ID NO: 19 - RNA, 2051 nt, synthetic construct
  source 1..2051: mol_type = other RNA; note = gE2 120A mRNA
gagttaggagttggtggcagtttcaataacaggtcattgccgagaaaaggatagcactataatatgggcaccgtgaacaagcccgtggtgggcgtgctgatgggcttcggcatcatcaccggcaccctgcgcatcaccaaccccgtgcgggccagcgtgctgcgctacgacgacttccacatcgacgaggacaagctggacaccaactccgtgtacgagccctactaccacagcgaccacgccgagtccagctgggtgaaccggggcgagtccagccgcaaggcctacgaccacaactccccctacatctggccccggaacgactacgacggcttcctggagaacgcccacgagcaccacggggtgtacaaccagggccgcgggatcgacagcggcgagcggctgatgcagcccacccagatgtccgcccaggaggacctgggggacgacaccggcatccacgtgatccccaccctgaacggggacgaccgccacaagatcgtgaacgtggaccagcggcagtacggcgacgtgttcaagggggacctgaaccccaagccccagggccagcgcctgatcgaggtcagcgtggaggagaaccaccccttcaccctgcgggcccccatccagcgcatctacggggtccggtacaccgagacctggtccttcctgcccagcctgacctgcaccggcgacgccgcccccgccatccagcacatctgcctgaagcacaccacctgcttccaggacgtggtcgtggacgtcgactgcgccgagaacaccaaggaggaccagctcgccgagatctcctaccgcttccaggggaagaaggaggccgaccagccctggatcgtggtcaacaccagcaccctgttcgacgagctggagctggacccgcccgagatcgagcccggcgtgctcaaggtcctgcggaccgagaagcagtacctcggggtgtacatctggaacatgcgcggctccgacgggaccagcacctacgccaccttcctggtcacctggaagggcgacgagaagacccggaaccccacccccgccgtgacgccccagccgcgcggggccgagttccacatgtggaactaccactcccacgtcttcagcgtgggcgacacgttctccctcgccatgcacctgcagtacaagatccacgaggccccgttcgacctcctgctggagtggctgtacgtccccatcgacccgacctgccagcccatgcggctctacagcacgtgcctgtaccaccccaacgccccgcagtgcctctcccacatgaacagcgggtgcaccttcacgtccccgcacctggcgcagcgcgtggccagcaccgtctaccagaactgcgagcacgcggacaactacaccgcctactgcctcggcatctcccacatggagccctcgttcgggctgatcctccacgacggcgggacgaccctgaagttcgtggacacgccggagagcctctccggcctgtacgtcttcgtggtctacttcaacgggcacgtggaggcggtcgcctacacggtggtctcgaccgtggaccacttcgtcaacgcgatcgaggagcggggctttcccccgaccgccgggcagccgcccgcgacgacgaagccgaaggagatcaccccggtgaaccccggcacgagcccgctcctgcgctacgccgcgtggaccgggggcctcgccgcggtcgtgctgctctgcctggtcatcttcctcatctgcaccgccaagcggatgcgcgtgaaggcggcccgggtcgacaagtcctgatgaaccggtgctcgctttcttgctgtccaatttctattaaaggttcctttgttccctaagtccaactactaaactgggggatattatgaagggccttgagcatctggattctgcctaataaaaaacatttattttcattgcaaaaaaaaaaaaaaaaaaaaaaaaaaaaaaaaaaaaaaaaaaaaaaaaaaaaaaaaaaaaaaaaaaaaaaaaaaaaaaaaaaaaaaaaaaaaaaaaaaaaaaaaaaaaaaaaaaaaaaaaaa

SEQ ID NO: 20 - RNA, 2198 nt, synthetic construct
  source 1..2198: mol_type = other RNA; note = gE6 120A mRNA
gagttaggagttggtggcagtttcaataacaggtcattgccgagaaaaggatagcactataatatgggcaccgtgaacaagcccgtggtgggcgtgctgatgggcttcggcatcatcaccggcaccctgcgcatcaccaaccccgtgcgggccagcgtgctgcgctacgacgacttccacatcgacgaggacaagctggacaccaactccgtgtacgagccctactaccacagcgaccacgccgagtccagctgggtgaaccggggcgagtccagccgcaaggcctacgaccacaactccccctacatctggccccggaacgactacgacggcttcctggagaacgcccacgagcaccacggggtgtacaaccagggccgcgggatcgacagcggcgagcggctgatgcagcccacccagatgtccgcccaggaggacctgggggacgacaccggcatccacgtgatccccaccctgaacggggacgaccgccacaagatcgtgaacgtggaccagcggcagtacggcgacgtgttcaagggggacctgaaccccaagccccagggccagcgcctgatcgaggtcagcgtggaggagaaccaccccttcaccctgcgggcccccatccagcgcatctacggggtccggtacaccgagacctggtccttcctgcccagcctgacctgcaccggcgacgccgcccccgccatccagcacatctgcctgaagcacaccacctgcttccaggacgtggtcgtggacgtcgactgcgccgagaacaccaaggaggaccagctcgccgagatctcctaccgcttccaggggaagaaggaggccgaccagccctggatcgtggtcaacaccagcaccctgttcgacgagctggagctggacccgcccgagatcgagcccggcgtgctcaaggtcctgcggaccgagaagcagtacctcggggtgtacatctggaacatgcgcggctccgacgggaccagcacctacgccaccttcctggtcacctggaagggcgacgagaagacccggaaccccacccccgccgtgacgccccagccgcgcggggccgagttccacatgtggaactaccactcccacgtcttcagcgtgggcgacacgttctccctcgccatgcacctgcagtacaagatccacgaggccccgttcgacctcctgctggagtggctgtacgtccccatcgacccgacctgccagcccatgcggctctacagcacgtgcctgtaccaccccaacgccccgcagtgcctctcccacatgaacagcgggtgcaccttcacgtccccgcacctggcgcagcgcgtggccagcaccgtctaccagaactgcgagcacgcggacaactacaccgcctactgcctcggcatctcccacatggagccctcgttcgggctgatcctccacgacggcgggacgaccctgaagttcgtggacacgccggagagcctctccggcctgtacgtcttcgtggtctacttcaacgggcacgtggaggcggtcgcctacacggtggtctcgaccgtggaccacttcgtcaacgcgatcgaggagcggggctttcccccgaccgccgggcagccgcccgcgacgacgaagccgaaggagatcaccccggtgaaccccggcacgagcccgctcctgcgctacgccgcgtggaccgggggcctcgccgcggtcgtgctgctctgcctggtcatcttcctcatctgcaccgccaagcggatgcgcgtgaaggcgtaccgggtcgacaagtccccctacaaccagtcgatgtactacgccgggctgcccgtggacgacttcgaggacagcgagtccacggacaccgaggaggagttcggcaacgcgatcgggggctcgcacgggggctcctcgtacacggtctacatcgacaagacccgctgatgaaccggtgctcgctttcttgctgtccaatttctattaaaggttcctttgttccctaagtccaactactaaactgggggatattatgaagggccttgagcatctggattctgcctaataaaaaacatttattttcattgcaaaaaaaaaaaaaaaaaaaaaaaaaaaaaaaaaaaaaaaaaaaaaaaaaaaaaaaaaaaaaaaaaaaaaaaaaaaaaaaaaaaaaaaaaaaaaaaaaaaaaaaaaaaaaaaaaaaaaaaaaa

SEQ ID NO: 21 - protein, 546 aa, synthetic construct
  source 1..546: note = gE1
MGTVNKPVVGVLMGFGIITGTLRITNPVRASVLRYDDFHIDEDKLDTNSVYEPYYHSDHAESSWVNRGESSRKAYDHNSPYIWPRNDYDGFLENAHEHHGVYNQGRGIDSGERLMQPTQMSAQEDLGDDTGIHVIPTLNGDDRHKIVNVDQRQYGDVFKGDLNPKPQGQRLIEVSVEENHPFTLRAPIQRIYGVRYTETWSFLPSLTCTGDAAPAIQHICLKHTTCFQDVVVDVDCAENTKEDQLAEISYRFQGKKEADQPWIVVNTSTLFDELELDPPEIEPGVLKVLRTEKQYLGVYIWNMRGSDGTSTYATFLVTWKGDEKTRNPTPAVTPQPRGAEFHMWNYHSHVFSVGDTFSLAMHLQYKIHEAPFDLLLEWLYVPIDPTCQPMRLYSTCLYHPNAPQCLSHMNSGCTFTSPHLAQRVASTVYQNCEHADNYTAYCLGISHMEPSFGLILHDGGTTLKFVDTPESLSGLYVFVVYFNGHVEAVAYTVVSTVDHFVNAIEERGFPPTAGQPPATTKPKEITPVNPGTSPLLRYAAWTGGLA

SEQ ID NO: 22 - protein, 574 aa, synthetic construct
  source 1..574: note = gE2
MGTVNKPVVGVLMGFGIITGTLRITNPVRASVLRYDDFHIDEDKLDTNSVYEPYYHSDHAESSWVNRGESSRKAYDHNSPYIWPRNDYDGFLENAHEHHGVYNQGRGIDSGERLMQPTQMSAQEDLGDDTGIHVIPTLNGDDRHKIVNVDQRQYGDVFKGDLNPKPQGQRLIEVSVEENHPFTLRAPIQRIYGVRYTETWSFLPSLTCTGDAAPAIQHICLKHTTCFQDVVVDVDCAENTKEDQLAEISYRFQGKKEADQPWIVVNTSTLFDELELDPPEIEPGVLKVLRTEKQYLGVYIWNMRGSDGTSTYATFLVTWKGDEKTRNPTPAVTPQPRGAEFHMWNYHSHVFSVGDTFSLAMHLQYKIHEAPFDLLLEWLYVPIDPTCQPMRLYSTCLYHPNAPQCLSHMNSGCTFTSPHLAQRVASTVYQNCEHADNYTAYCLGISHMEPSFGLILHDGGTTLKFVDTPESLSGLYVFVVYFNGHVEAVAYTVVSTVDHFVNAIEERGFPPTAGQPPATTKPKEITPVNPGTSPLLRYAAWTGGLAAVVLLCLVIFLICTAKRMRVKAARVDKS

SEQ ID NO: 23 - protein, 544 aa, synthetic construct
  source 1..544: note = gE3
MGTVNKPVVGVLMGFGIITGTLRITNPVRASVLRYDDFHIDEDKLDTNSVYEPYYHSDHAESSWVNRGESSRKAYDHNSPYIWPRNDYDGFLENAHEHHGVYNQGRGIDSGERLMQPTQMSAQEDLGDDTGIHVIPTLNGDDRHKIVNVDQRQYGDVFKGDLNPKPQGQRLIEVSVEENHPFTLRAPIQRIYGVRYTETWSFLPSLTCTGDAAPAIQHICLKHTTCFQDVVVDVDCAENTKEDQLAEISYRFQGKKEADQPWIVVNTSTLFDELELDPPEIEPGVLKVLRTEKQYLGVYIWNMRGSDGTSTYATFLVTWKGDEKTRNPTPAVTPQPRGAEFHMWNYHSHVFSVGDTFSLAMHLQYKIHEAPFDLLLEWLYVPIDPTCQPMRLYSTCLYHPNAPQCLSHMNSGCTFTSPHLAQRVASTVYQNCEHADNYTAYCLGISHMEPSFGLILHDGGTTLKFVDTPESLSGLYVFVVYFNGHVEAVAYTVVSTVDHFVNAIEERGFPPTAGQPPATTKPKEITPVNPGTSPLLRYAAWTGG

SEQ ID NO: 24 - protein, 574 aa, synthetic construct
  source 1..574: note = gE4
MGTVNKPVVGVLMGFGIITGTLRITNPVRASVLRYDDFHIDEDKLDTNSVYEPYYHSDHAESSWVNRGESSRKAYDHNSPYIWPRNDYDGFLENAHEHHGVYNQGRGIDSGERLMQPTQMSAQEDLGDDTGIHVIPTLNGDDRHKIVNVDQRQYGDVFKGDLNPKPQGQRLIEVSVEENHPFTLRAPIQRIYGVRYTETWSFLPSLTCTGDAAPAIQHICLKHTTCFQDVVVDVDCAENTKEDQLAEISYRFQGKKEADQPWIVVNTSTLFDELELDPPEIEPGVLKVLRTEKQYLGVYIWNMRGSDGTSTYATFLVTWKGDEKTRNPTPAVTPQPRGAEFHMWNYHSHVFSVGDTFSLAMHLQYKIHEAPFDLLLEWLYVPIDPTCQPMRLYSTCLYHPNAPQCLSHMNSGCTFTSPHLAQRVASTVYQNCEHADNYTAYCLGISHMEPSFGLILHDGGTTLKFVDTPESLSGLYVFVVYFNGHVEAVAYTVVSTVDHFVNAIEERGFPPTAGQPPATTKPKEITPVNPGTSPLLRYAAWTGGLAAVVLLCLVIFLICTAKRMRVKAYRVDKS

SEQ ID NO: 25 - protein, 561 aa, synthetic construct
  source 1..561: note = gE5
MGTVNKPVVGVLMGFGIITGTLRITNPVRASVLRYDDFHIDEDKLDTNSVYEPYYHSDHAESSWVNRGESSRKAYDHNSPYIWPRNDYDGFLENAHEHHGVYNQGRGIDSGERLMQPTQMSAQEDLGDDTGIHVIPTLNGDDRHKIVNVDQRQYGDVFKGDLNPKPQGQRLIEVSVEENHPFTLRAPIQRIYGVRYTETWSFLPSLTCTGDAAPAIQHICLKHTTCFQDVVVDVDCAENTKEDQLAEISYRFQGKKEADQPWIVVNTSTLFDELELDPPEIEPGVLKVLRTEKQYLGVYIWNMRGSDGTSTYATFLVTWKGDEKTRNPTPAVTPQPRGAEFHMWNYHSHVFSVGDTFSLAMHLQYKIHEAPFDLLLEWLYVPIDPTCQPMRLYSTCLYHPNAPQCLSHMNSGCTFTSPHLAQRVASTVYQNCEHADNYTAYCLGISHMEPSFGLILHDGGTTLKFVDTPESLSGLYVFVVYFNGHVEAVAYTVVSTVDHFVNAIEERGFPPTAGQPPATTKPKEITPVNPGTSPLLRYAAWTGGLAAVVLLCLVIFLICTA

SEQ ID NO: 26 - RNA, 2130 nt, synthetic construct
  source 1..2130: mol_type = other RNA; note; note (original language) = 荧光素酶
taatacgactcactataagggaagcttctctcgcactctgttcttccgccgctccgccgtcgcgtttctctgccggtcgcagctagccttaaggccaccatggaagacgccaaaaacataaagaaaggcccggcgccattctatccgctggaagatggaaccgctggagagcaactgcataaggctatgaagagatacgccctggttcctggaacaattgcttttacagatgcacatatcgaggtggacatcacttacgctgagtacttcgaaatgtccgttcggttggcagaagctatgaaacgatatgggctgaatacaaatcacagaatcgtcgtatgcagtgaaaactctcttcaattctttatgccggtgttgggcgcgttatttatcggagttgcagttgcgcccgcgaacgacatttataatgaacgtgaattgctcaacagtatgggcatttcgcagcctaccgtggtgttcgtttccaaaaaggggttgcaaaaaattttgaacgtgcaaaaaaagctcccaatcatccaaaaaattattatcatggattctaaaacggattaccagggatttcagtcgatgtacacgttcgtcacatctcatctacctcccggttttaatgaatacgattttgtgccagagtccttcgatagggacaagacaattgcactgatcatgaactcctctggatctactggtctgcctaaaggtgtcgctctgcctcatagaactgcctgcgtgagattctcgcatgccagagatcctatttttggcaatcaaatcattccggatactgcgattttaagtgttgttccattccatcacggttttggaatgtttactacactcggatatttgatatgtggatttcgagtcgtcttaatgtatagatttgaagaagagctgtttctgaggagccttcaggattacaagattcaaagtgcgctgctggtgccaaccctattctccttcttcgccaaaagcactctgattgacaaatacgatttatctaatttacacgaaattgcttctggtggcgctcccctctctaaggaagtcggggaagcggttgccaagaggttccatctgccaggtatcaggcaaggatatgggctcactgagactacatcagctattctgattacacccgagggggatgataaaccgggcgcggtcggtaaagttgttccattttttgaagcgaaggttgtggatctggataccgggaaaacgctgggcgttaatcaaagaggcgaactgtgtgtgagaggtcctatgattatgtccggttatgtaaacaatccggaagcgaccaacgccttgattgacaaggatggatggctacattctggagacatagcttactgggacgaagacgaacacttcttcatcgttgaccgcctgaagtctctgattaagtacaaaggctatcaggtggctcccgctgaattggaatccatcttgctccaacaccccaacatcttcgacgcaggtgtcgcaggtcttcccgacgatgacgccggtgaacttcccgccgccgttgttgttttggagcacggaaagacgatgacggaaaaagagatcgtggattacgtcgccagtcaagtaacaaccgcgaaaaagttgcgcggaggagttgtgtttgtggacgaagtaccgaaaggtcttaccggaaaactcgacgcaagaaaaatcagagagatcctcataaaggccaagaagggcggaaagatcgccgtggattacaaggatgacgacgataagtaagggccctctgccgtgggcctgtcgtgccagtcctgggggcgagatcgggagaatcacgtcctggaactgcatgttcttgcgactcttgggacttcatcttaacttctcgctgccccagccatgttttcaaccatggcatccctcccccaattagttccctgtcatcctcgtcaaccttctctgtaagtgcctggtaagcttgcccttgcttaagaactcaaaacatagctgtgctctaccgcggaaaaaaaaaaaaaaaaaaaaaaaaaaaaaagcatatgactaaaaaaaaaaaaaaaaaaaaaaaaaaaaaaaaaaaaaaaaaaaaaaaaaaaaaaaaaaaaaaaaaaaaaa